European Patent Application EP 4 643 887 A1, published November 5, 2025. Title: 抗BDCA2抗体-药物偶联物及其用途. Applicant: 映恩生物制药（苏州）有限公司. The sequence listing filed with the application follows.

SEQUENCE LISTING (26 sequences)

SEQ ID NO: 1 - protein, 5 aa, synthetic construct
SYGMS

SEQ ID NO: 2 - protein, 17 aa, synthetic construct
TISSGDSYTYYPDSVKG

SEQ ID NO: 3 - protein, 12 aa, synthetic construct
QIYYDYAYYFDF

SEQ ID NO: 4 - protein, 15 aa, synthetic construct
RASESVSFRTSHLMH

SEQ ID NO: 5 - protein, 7 aa, synthetic construct
GASNLES

SEQ ID NO: 6 - protein, 9 aa, synthetic construct
QQSIEDPPT

SEQ ID NO: 7 - protein, 5 aa, synthetic construct
NYGVH

SEQ ID NO: 8 - protein, 16 aa, synthetic construct
VIWSGESTDYDAAFIS

SEQ ID NO: 9 - protein, 12 aa, synthetic construct
RRSHYYGYVMDY

SEQ ID NO: 10 - protein, 15 aa, synthetic construct
KASQSIDYDAIGYLN

SEQ ID NO: 11 - protein, 7 aa, synthetic construct
AASNLES

SEQ ID NO: 12 - protein, 9 aa, synthetic construct
QQSNEDPPT

SEQ ID NO: 13 - protein, 121 aa, synthetic construct
EVQLVESGGGLVKPGGSLRLSCAASGFTFSSYGMSWVRQAPGKGLEWVSTISSGDSYTYYPDSVKGRFTISRDNAKNSLYLQMNSLRAEDTAVYYCARQIYYDYAYYFDFWGQGTTVTVSS

SEQ ID NO: 14 - protein, 111 aa, synthetic construct
DIVLTQSPASLAVSPGQRATITCRASESVSFRTSHLMHWYQQKPGQPPKLLIYGASNLESGVPARFSGSGSETDFTLTINPVEAEDTANYFCQQSIEDPPTFGGGTKVEIK

SEQ ID NO: 15 - protein, 121 aa, synthetic construct
EVQLVESGGGLVKPGGSLRLSCAASGFTFRSYGMSWVRQAPGKRLEWVSTISSGDSYTYYPDSVKGRFTISRDNAKNSLYLQMNSLKAEDTAVYYCARQIYYDYAYYFDFWGQGTTVTVSS

SEQ ID NO: 16 - protein, 111 aa, synthetic construct
DIVMTQSPDSLAVSLGERATINCRASESVSFRTSHLMHWYQQKPGQPPKLLIYGASNLESGVPDRFSGSGSGTDFTLTISSLQAEDVAVYYCQQSIEDPPTFGGGTKVEIK

SEQ ID NO: 17 - protein, 120 aa, synthetic construct
QVQLQQSGPGLVKPSETLSLTCTVSGGSLTNYGVHWIRQPPGKGLEWIGVIWSGESTDYDAAFISRVTISKDNSKNQVSLKLSSVTAADTAVYYCARRRSHYYGYVMDYWGQGTTVTVSS

SEQ ID NO: 18 - protein, 111 aa, synthetic construct
DIVLTQSPASLAVSPGQRATITCKASQSIDYDAIGYLNWYQQKPGQPPKLLIYAASNLESGVPARFSGSGSGTDFTLTINPVEANDTANYYCQQSNEDPPTFGQGTKLEIK

SEQ ID NO: 19 - protein, 451 aa, synthetic construct
EVQLVESGGGLVKPGGSLRLSCAASGFTFSSYGMSWVRQAPGKGLEWVSTISSGDSYTYYPDSVKGRFTISRDNAKNSLYLQMNSLRAEDTAVYYCARQIYYDYAYYFDFWGQGTTVTVSSASTKGPSVFPLAPSSKSTSGGTAALGCLVKDYFPEPVTVSWNSGALTSGVHTFPAVLQSSGLYSLSSVVTVPSSSLGTQTYICNVNHKPSNTKVDKKVEPKSCDKTHTCPPCPAPELLGGPSVFLFPPKPKDTLMISRTPEVTCVVVDVSHEDPEVKFNWYVDGVEVHNAKTKPREEQYNSTYRVVSVLTVLHQDWLNGKEYKCKVSNKALPAPIEKTISKAKGQPREPQVYTLPPSRDELTKNQVSLTCLVKGFYPSDIAVEWESNGQPENNYKTTPPVLDSDGSFFLYSKLTVDKSRWQQGNVFSCSVMHEALHNHYTQKSLSLSPGK

SEQ ID NO: 20 - protein, 218 aa, synthetic construct
DIVLTQSPASLAVSPGQRATITCRASESVSFRTSHLMHWYQQKPGQPPKLLIYGASNLESGVPARFSGSGSETDFTLTINPVEAEDTANYFCQQSIEDPPTFGGGTKVEIKRTVAAPSVFIFPPSDEQLKSGTASVVCLLNNFYPREAKVQWKVDNALQSGNSQESVTEQDSKDSTYSLSSTLTLSKADYEKHKVYACEVTHQGLSSPVTKSFNRGEC

SEQ ID NO: 21 - protein, 451 aa, synthetic construct
EVQLVESGGGLVKPGGSLRLSCAASGFTFRSYGMSWVRQAPGKRLEWVSTISSGDSYTYYPDSVKGRFTISRDNAKNSLYLQMNSLKAEDTAVYYCARQIYYDYAYYFDFWGQGTTVTVSSASTKGPSVFPLAPSSKSTSGGTAALGCLVKDYFPEPVTVSWNSGALTSGVHTFPAVLQSSGLYSLSSVVTVPSSSLGTQTYICNVNHKPSNTKVDKKVEPKSCDKTHTCPPCPAPELLGGPSVFLFPPKPKDTLMISRTPEVTCVVVDVSHEDPEVKFNWYVDGVEVHNAKTKPREEQYNSTYRVVSVLTVLHQDWLNGKEYKCKVSNKALPAPIEKTISKAKGQPREPQVYTLPPSRDELTKNQVSLTCLVKGFYPSDIAVEWESNGQPENNYKTTPPVLDSDGSFFLYSKLTVDKSRWQQGNVFSCSVMHEALHNHYTQKSLSLSPGK

SEQ ID NO: 22 - protein, 218 aa, synthetic construct
DIVMTQSPDSLAVSLGERATINCRASESVSFRTSHLMHWYQQKPGQPPKLLIYGASNLESGVPDRFSGSGSGTDFTLTISSLQAEDVAVYYCQQSIEDPPTFGGGTKVEIKRTVAAPSVFIFPPSDEQLKSGTASVVCLLNNFYPREAKVQWKVDNALQSGNSQESVTEQDSKDSTYSLSSTLTLSKADYEKHKVYACEVTHQGLSSPVTKSFNRGEC

SEQ ID NO: 23 - protein, 450 aa, synthetic construct
QVQLQQSGPGLVKPSETLSLTCTVSGGSLTNYGVHWIRQPPGKGLEWIGVIWSGESTDYDAAFISRVTISKDNSKNQVSLKLSSVTAADTAVYYCARRRSHYYGYVMDYWGQGTTVTVSSASTKGPSVFPLAPSSKSTSGGTAALGCLVKDYFPEPVTVSWNSGALTSGVHTFPAVLQSSGLYSLSSVVTVPSSSLGTQTYICNVNHKPSNTKVDKKVEPKSCDKTHTCPPCPAPELLGGPSVFLFPPKPKDTLMISRTPEVTCVVVDVSHEDPEVKFNWYVDGVEVHNAKTKPREEQYNSTYRVVSVLTVLHQDWLNGKEYKCKVSNKALPAPIEKTISKAKGQPREPQVYTLPPSRDELTKNQVSLTCLVKGFYPSDIAVEWESNGQPENNYKTTPPVLDSDGSFFLYSKLTVDKSRWQQGNVFSCSVMHEALHNHYTQKSLSLSPGK

SEQ ID NO: 24 - protein, 218 aa, synthetic construct
DIVLTQSPASLAVSPGQRATITCKASQSIDYDAIGYLNWYQQKPGQPPKLLIYAASNLESGVPARFSGSGSGTDFTLTINPVEANDTANYYCQQSNEDPPTFGQGTKLEIKRTVAAPSVFIFPPSDEQLKSGTASVVCLLNNFYPREAKVQWKVDNALQSGNSQESVTEQDSKDSTYSLSSTLTLSKADYEKHKVYACEVTHQGLSSPVTKSFNRGEC

SEQ ID NO: 25 - protein, 451 aa, synthetic construct
DVQLVESGGGLVKPGGSLRLSCAASGFTFSTYTMSWVRQAPGKGLEWVATISPGDSFGYYYPDSVQGRFTISRDNAKNSLYLQMNSLRAEDTAVYYCTRDIYYNYGAWFAYWGQGTLVTVSSASTKGPSVFPLAPSSKSTSGGTAALGCLVKDYFPEPVTVSWNSGALTSGVHTFPAVLQSSGLYSLSSVVTVPSSSLGTQTYICNVNHKPSNTKVDKKVEPKSCDKTHTCPPCPAPELLGGPSVFLFPPKPKDTLMISRTPEVTCVVVDVSHEDPEVKFNWYVDGVEVHNAKTKPREEQYNSTYRVVSVLTVLHQDWLNGKEYKCKVSNKALPAPIEKTISKAKGQPREPQVYTLPPSRDELTKNQVSLTCLVKGFYPSDIAVEWESNGQPENNYKTTPPVLDSDGSFFLYSKLTVDKSRWQQGNVFSCSVMHEALHNHYTQKSLSLSPG

SEQ ID NO: 26 - protein, 218 aa, synthetic construct
DIQLTQSPSSLSASVGDRVTITCKASQSVDYDGDSYMNWYQQKPGKAPKLLIYAASTLESGVPSRFSGSGSGTDFTLTISSLQPEDFATYYCQQANEDPRTFGQGTKVEIKRTVAAPSVFIFPPSDEQLKSGTASVVCLLNNFYPREAKVQWKVDNALQSGNSQESVTEQDSKDSTYSLSSTLTLSKADYEKHKVYACEVTHQGLSSPVTKSFNRGEC